European Patent Application EP 4 692 114 A1, published February 11, 2026. Title: 一种降钙素类似物及其衍生物和用途. Applicant: 杭州先为达生物科技股份有限公司. The sequence listing filed with the application follows.

SEQUENCE LISTING (38 sequences)

SEQ ID NO: 1 - protein, 37 aa, synthetic construct
KCNTATCATQRLAEFLRHSSNNFGPILPPTNVGSNTP

SEQ ID NO: 2 - protein, 32 aa, synthetic construct
CSNLSTCVLGKLSQELHKLQTYPRTNTGSGTP

SEQ ID NO: 3 - protein, 33 aa, synthetic construct
EASELSTAALGRLSAELHELATLPRTETGPESP

SEQ ID NO: 4 - protein, 31 aa, synthetic construct
HVEGTFTSDVSSYLEEQAAREFIKWLVRGRG

SEQ ID NO: 5 - protein, 32 aa, synthetic construct
ASQLSTAVLGRLSQELHRLQDYPRTDVGSGSP

SEQ ID NO: 6 - protein, 32 aa, synthetic construct
ASDLSTAVLGRLSQELHRLQDYPRTDVGSGSP

SEQ ID NO: 7 - protein, 32 aa, synthetic construct
ASQLSTAVLGRLSDELHRLQDYPRTDVGSGSP

SEQ ID NO: 8 - protein, 32 aa, synthetic construct
ASQLSTAVLGRLSEELHRLQDYPRTDVGSGSP

SEQ ID NO: 9 - protein, 34 aa, synthetic construct
ASQLSTAVLGRLSAIBELHRLQDYPRTDVGSGSP

SEQ ID NO: 10 - protein, 32 aa, synthetic construct
ASQLSTAVLGRLSSELHRLQDYPRTDVGSGSP

SEQ ID NO: 11 - protein, 32 aa, synthetic construct
ASQLSTAVLGRLSTELHRLQDYPRTDVGSGSP

SEQ ID NO: 12 - protein, 32 aa, synthetic construct
ASQLSTAVLGRLSQELHRLEDYPRTDVGSGSP

SEQ ID NO: 13 - protein, 32 aa, synthetic construct
ASQLSTAVLGRLSQELHRLEEYPRTDVGSGSP

SEQ ID NO: 14 - protein, 32 aa, synthetic construct
ASQLSTAVLGRLSQELHRLQDYPRTQVGSGSP

SEQ ID NO: 15 - protein, 32 aa, synthetic construct
ASQLSTAVLGRLSQELHRLQDYPRTDSGSGSP

SEQ ID NO: 16 - protein, 32 aa, synthetic construct
ASQLSTAVLGRLSQELHRLQDYPRTQSGSGSP

SEQ ID NO: 17 - protein, 32 aa, synthetic construct
ASQLSTAVLGRLSQELHRLQDLPRTDVGSGSP

SEQ ID NO: 18 - protein, 32 aa, synthetic construct
ASQLSTAVLGRLSQELHRLQDYPRTDVGAGSP

SEQ ID NO: 19 - protein, 32 aa, synthetic construct
ASQLSTAVLGRLSQELHRLQDYPRTDVGAESP

SEQ ID NO: 20 - protein, 32 aa, synthetic construct
ASQLSTAVLGRLSQELHRLQDYPRTDVGSESP

SEQ ID NO: 21 - protein, 32 aa, synthetic construct
  MOD_RES 32: note = trans-Hyp -NH2
ASQLSTAVLGRLSQELHRLQDYPRTDVGSGSX

SEQ ID NO: 22 - protein, 33 aa, synthetic construct
DASQLSTAVLGRLSQELHRLQDYPRTDVGSGSP

SEQ ID NO: 23 - protein, 33 aa, synthetic construct
EASQLSTAVLGRLSQELHRLQDYPRTDVGSGSP

SEQ ID NO: 24 - protein, 32 aa, synthetic construct
LSQLSTLVLGRLSQELHRLQDYPRTDVGSGSP

SEQ ID NO: 25 - protein, 32 aa, synthetic construct
VSQLSTVVLGRLSQELHRLQDYPRTDVGSGSP

SEQ ID NO: 26 - protein, 32 aa, synthetic construct
ISQLSTIVLGRLSQELHRLQDYPRTDVGSGSP

SEQ ID NO: 27 - protein, 32 aa, synthetic construct
SSQLSTSVLGRLSQELHRLQDYPRTDVGSGSP

SEQ ID NO: 28 - protein, 32 aa, synthetic construct
ASQLSTSVLGRLSQELHRLQDYPRTDVGSGSP

SEQ ID NO: 29 - protein, 32 aa, synthetic construct
SSQLSTAVLGRLSQELHRLQDYPRTDVGSGSP

SEQ ID NO: 30 - protein, 32 aa, synthetic construct
ESQLSTRVLGRLSQELHRLQDYPRTDVGSGSP

SEQ ID NO: 31 - protein, 32 aa, synthetic construct
RSQLSTEVLGRLSQELHRLQDYPRTDVGSGSP

SEQ ID NO: 32 - protein, 32 aa, synthetic construct
ESQLSTEVLGRLSQELHRLQDYPRTDVGSGSP

SEQ ID NO: 33 - protein, 32 aa, synthetic construct
ASELSTAVLGRLSEELHRLEDYPRTDVGSGSP

SEQ ID NO: 34 - protein, 32 aa, synthetic construct
RSQLSTDVLGRLSQELHRLQDYPRTDVGSGSP

SEQ ID NO: 35 - protein, 32 aa, synthetic construct
KSQLSTEVLGRLSQELHRLQDYPRTDVGSGSP

SEQ ID NO: 36 - protein, 32 aa, synthetic construct
KSQLSTDVLGRLSQELHRLQDYPRTDVGSGSP

SEQ ID NO: 37 - protein, 32 aa, synthetic construct
ASQLSTAVLGRLSQELHRLQDFPRTDVGSGSP

SEQ ID NO: 38 - protein, 32 aa, synthetic construct
ASQLSTAVLGRLSDELHRLQDLPRTDVGSGSP